European Patent Specification EP 3 878 971 B1, published December 4, 2024. Title: PROCÉDÉ POUR DÉTECTER ET ÉVENTUELLEMENT QUANTIFIER UN ANALYTE AVEC UN OLIGONUCLÉOTIDE À DOUBLE STRUCTURE TIGE-BOUCLE ET LEDIT OLIGONUCLÉOTIDE. Applicant: Commissariat à l'Energie Atomique et aux Energies Renouvelables (CEA) Centre National de la Recherche Scientifique (CNRS) Université Grenoble Alpes (UGA). Application EP20XXXXX. The sequence listing filed with the application follows.

SEQUENCE LISTING (10 sequences)

SEQ ID NO: 1 - DNA, 63 bp, Unknown
  Séquence artificielle
  misc_feature (1)..(63): ADN cible à détecter désigné Tro4cZip6
taagaggggcagcgcatgagaaaggttggcgtactgcacggaccggtatgcgacctggtatgc

SEQ ID NO: 2 - DNA, 24 bp, Unknown
  Séquence artificielle
  misc_feature (1)..(24): Sonde ADN biotinylée désignée Zip6cbio
cgcataccaggtcgcataccggtc

SEQ ID NO: 3 - DNA, 153 bp, Unknown
  Séquence artificielle
  misc_feature (1)..(153): Oligonucléotide à double structure tige-boucle de formule (I)
cggatccaagacgcggtttatcgtgcagtacgccaacctttctcatgcgctgcccctcttaataaaccgcgtcttggatccgtgacatctctgagttatatctttccccccctcactgaccctccttcgggggaaagatataactcagagatg

SEQ ID NO: 4 - DNA, 45 bp, Unknown
  Séquence artificielle
  misc_feature (1)..(45): Amorce FIP
cggatccaagacgcggtttatcgtgcagtacgccaacctttctca

SEQ ID NO: 5 - DNA, 43 bp, Unknown
  Séquence Artificielle
  misc_feature (1)..(43): Amorce BIP
catctctgagttatatctttcccccgaaggagggtcagtgagg

SEQ ID NO: 6 - DNA, 42 bp, Unknown
  Séquence artificielle
  misc_feature (1)..(42): ADN cible à détecter
gaaggagggtcagtgagggaccggtatgcgacctggtatgcg

SEQ ID NO: 7 - DNA, 134 bp, Unknown
  Séquence artificielle
  misc_feature (1)..(134): Oligonucléotide à double structure tige-boucle de formule (II)
cggatccaagacgcggtttatcgtgcagtacgccaacctttctcaataaaccgcgtcttggatccgcatctctgagttatatctttccccccctcactgaccctccttcgggggaaagatataactcagagatg

SEQ ID NO: 8 - DNA, 15 bp, Unknown
  Séquence artificielle
  misc_feature (1)..(15): Aptamère Thr1
ggttggtgtggttgg

SEQ ID NO: 9 - DNA, 29 bp, Unknown
  Séquence artificielle
  misc_feature (1)..(29): Aptamère Thr2
agtccgtggtagggcaggttggggtgact

SEQ ID NO: 10 - DNA, 152 bp, Unknown
  Séquence artificielle
  misc_feature (1)..(152): Oligonucléotide à double structure tige-boucle DTRC
cggatccaagacgcggtttatcgtgcagtacgccaacctttctcaataaaccgcgtcttggatccgtggttggtgtggttgggacatctctgagttatatctttccccccctcactgaccctccttcgggggaaagatataactcagagatg